European Patent Application EP 4 242 303 A1, published September 13, 2023. Title: Fusion polypeptides with deamidase inhibitor and deamidase domains. Applicant: Novozymes A/S. The sequence listing filed with the application follows.

SEQUENCE LISTING (25 sequences)

SEQ ID NO: 1 - DNA, 327 bp, Chryseobacterium sp-62563
  CDS (1)..(327)
aatcaggatccgaatcttgtagcaaaagagtctaacgaaactgctatgaaagatttcggcaagaccgtcccggtagggatcgagaaagaagatggaaaatttaaaatctcttttatggttactgcccagccttatgaaattaaggacagtaaagaaaatgcagcttatatttccatgatcaaaacggctgttgagaacgaaacacctattcatgttttcctgaaggccaatactaacgaaatagcaaaagtagacaaagcaacagatgatgacatccgttatttcaaatctgtcttcaccaaagaagtaaaagaagaaaacaggaaa

SEQ ID NO: 2 - protein, 109 aa, Chryseobacterium sp-62563
NQDPNLVAKESNETAMKDFGKTVPVGIEKEDGKFKISFMVTAQPYEIKDSKENAAYISMIKTAVENETPIHVFLKANTNEIAKVDKATDDDIRYFKSVFTKEVKEENRK

SEQ ID NO: 3 - DNA, 555 bp, Chryseobacterium sp-62563
  CDS (1)..(555)
gcggtaagtgttattcctaacctggccactttaaacagtctgtttgcccaaatcaaaaatcaggcttgcggaacttctacggcatcttcaccatgtatcacattcagatatcctgttgatggctgctatgcaagagctcacaaaatgagacaaatattactgaatgcaggttacgactgtgaaaaacagttcgtatatggtaacctgagagcttctacaggaacttgctgtgtatcttgggtatatcacgtagcaatattggtaagctttaagaatgcttcaggagttgttgagaaaagaatcatagatccttcattattctcaagcggacctgttactgatgctgcatggagagctgcatgtaccaataccagctgtggatctgcttctgtatcttctttcgccaatacggcaggaaatgtttactacagaagtccgtcaggatctttattgtatgataacaattatgtaaataccaactgtgtattgaatatattttcatccctatcaggatgttcaccttctcctgcacctagtgtagctagctgtggattt

SEQ ID NO: 4 - protein, 185 aa, Chryseobacterium sp-62563
AVSVIPNLATLNSLFAQIKNQACGTSTASSPCITFRYPVDGCYARAHKMRQILLNAGYDCEKQFVYGNLRASTGTCCVSWVYHVAILVSFKNASGVVEKRIIDPSLFSSGPVTDAAWRAACTNTSCGSASVSSFANTAGNVYYRSPSGSLLYDNNYVNTNCVLNIFSSLSGCSPSPAPSVASCGF

SEQ ID NO: 5 - protein, 294 aa, Chryseobacterium sp-62563
NQDPNLVAKESNETAMKDFGKTVPVGIEKEDGKFKISFMVTAQPYEIKDSKENAAYISMIKTAVENETPIHVFLKANTNEIAKVDKATDDDIRYFKSVFTKEVKEENRKAVSVIPNLATLNSLFAQIKNQACGTSTASSPCITFRYPVDGCYARAHKMRQILLNAGYDCEKQFVYGNLRASTGTCCVSWVYHVAILVSFKNASGVVEKRIIDPSLFSSGPVTDAAWRAACTNTSCGSASVSSFANTAGNVYYRSPSGSLLYDNNYVNTNCVLNIFSSLSGCSPSPAPSVASCGF

SEQ ID NO: 6 - DNA, 327 bp, Chryseobacterium gambrini
  CDS (1)..(327)
aatcaggatccgaatcttgttgtaaaagaaaacaatgaaaatgccatgagagactttggcagcactattccggtagggattcaaaaagaaggcaatgtcctgaaagtttctttcatcatttctgcgcagttctatgaaattaaagacagtaaagaaaatgaagccttcatctcaatgattaaatcagcaatagaaaatgaaactccggttcatgttttcctgaaaaaaaattccaacgaaattgccaaagttgaaaaagcaacagatgaagatgttacttacttcaaatccatcttcaccaaagaagtaaaagaagaaaacaggaaa

SEQ ID NO: 7 - protein, 109 aa, Chryseobacterium gambrini
NQDPNLVVKENNENAMRDFGSTIPVGIQKEGNVLKVSFIISAQFYEIKDSKENEAFISMIKSAIENETPVHVFLKKNSNEIAKVEKATDEDVTYFKSIFTKEVKEENRK

SEQ ID NO: 8 - DNA, 573 bp, Chryseobacterium gambrini
  CDS (1)..(573)
gcagtaagtgtaattccgaatctggcgactctgaacaatcttttcatacagatcaaaaatcagtcgtgcggaacttctacagcttcttcaccatgtatcacgttcagatatgcagtggacggatgttatgcaagagctcataaaatgagacagatccttctgaatgcaggttatgactgcgaaaaacaattcgtctacggaaacctgaaagcttctacaggaacgtgctgtgtttcgtggggatatcacgtagctattttagtaagctttaaaaatgcttccggtgtggttgaaaaaagaattatagatccttctcttttcacctccggaccggtaactgatactgcatggagaaatgcgtgcgtaaatacaagctgtggttccgcctctgcttcttcttacgccaatacggcaggaaatgtatattacagaagtccgtccggttcgctgctttatgacaacaattatataaacacgaattgtgtactgacaacattttctacattatccggatgctctccagttccggctccaagtgtagcaagctgtggattccatcatcaccatcaccac

SEQ ID NO: 9 - protein, 191 aa, Chryseobacterium gambrini
AVSVIPNLATLNNLFIQIKNQSCGTSTASSPCITFRYAVDGCYARAHKMRQILLNAGYDCEKQFVYGNLKASTGTCCVSWGYHVAILVSFKNASGVVEKRIIDPSLFTSGPVTDTAWRNACVNTSCGSASASSYANTAGNVYYRSPSGSLLYDNNYINTNCVLTTFSTLSGCSPVPAPSVASCGFHHHHHH

SEQ ID NO: 10 - protein, 300 aa, Chryseobacterium gambrini
NQDPNLVVKENNENAMRDFGSTIPVGIQKEGNVLKVSFIISAQFYEIKDSKENEAFISMIKSAIENETPVHVFLKKNSNEIAKVEKATDEDVTYFKSIFTKEVKEENRKAVSVIPNLATLNNLFIQIKNQSCGTSTASSPCITFRYAVDGCYARAHKMRQILLNAGYDCEKQFVYGNLKASTGTCCVSWGYHVAILVSFKNASGVVEKRIIDPSLFTSGPVTDTAWRNACVNTSCGSASASSYANTAGNVYYRSPSGSLLYDNNYINTNCVLTTFSTLSGCSPVPAPSVASCGFHHHHHH

SEQ ID NO: 11 - DNA, 327 bp, Chryseobacterium culicis
  CDS (1)..(327)
aatcaggatcccaatcttgttgctaaagagtctaatgaaatcgcgatgaaagatttcggtaaaactgttccggtagggattgaaaaagaagagggaaaatttaaagtctcttttatggtgagtgctcagccataccacattaaagacagtaaggaaaatgcaggttatatttctatgatcagacaagccgttgaaaacgaaactcctgttcatattttcctgaaaaccaacaccaatgaaattgcaaaagtagataaacctactgatgatgatatccgttatttcaaatctgttttcaccaaagaagtaaaagaagaaaacaggaaa

SEQ ID NO: 12 - protein, 109 aa, Chryseobacterium culicis
NQDPNLVAKESNEIAMKDFGKTVPVGIEKEEGKFKVSFMVSAQPYHIKDSKENAGYISMIRQAVENETPVHIFLKTNTNEIAKVDKPTDDDIRYFKSVFTKEVKEENRK

SEQ ID NO: 13 - DNA, 573 bp, Chryseobacterium culicis
  CDS (1)..(573)
gcagtgagtgttattcctaatctggcaacactgaacagcttatttacgcagattaaaaatcaggcttgtggtacttctacagcatcttctccatgtatcactttcagatatccagtggatggatgttatgcaagagctcacaaaatgagacaaattctccttaatgcaggttacgactgtgaaaagcagttcgtttacggaaacctgagagcttctacaggaacttgctgcgtatcatgggtatatcacgtagccatattggtaagcttcaaaaatgcttccggaattgttgagaaaagaatcatcgacccttcactattctccagcggacctgtaactgacgcagcatggagagccgcttgtaccaacacaagctgtggatctgcttctgtatcttcttttgccaatacagcaggaaatgtatattacagaagtccatcaggatctttactgtatgataacaattatgtaaataccaattgtgtattgaatatattctcatccctttcaggatgttctccttctcctgcaccaagtgtagcgagctgcggatttcatcatcaccatcaccac

SEQ ID NO: 14 - protein, 191 aa, Chryseobacterium culicis
AVSVIPNLATLNSLFTQIKNQACGTSTASSPCITFRYPVDGCYARAHKMRQILLNAGYDCEKQFVYGNLRASTGTCCVSWVYHVAILVSFKNASGIVEKRIIDPSLFSSGPVTDAAWRAACTNTSCGSASVSSFANTAGNVYYRSPSGSLLYDNNYVNTNCVLNIFSSLSGCSPSPAPSVASCGFHHHHHH

SEQ ID NO: 15 - protein, 300 aa, Chryseobacterium culicis
NQDPNLVAKESNEIAMKDFGKTVPVGIEKEEGKFKVSFMVSAQPYHIKDSKENAGYISMIRQAVENETPVHIFLKTNTNEIAKVDKPTDDDIRYFKSVFTKEVKEENRKAVSVIPNLATLNSLFTQIKNQACGTSTASSPCITFRYPVDGCYARAHKMRQILLNAGYDCEKQFVYGNLRASTGTCCVSWVYHVAILVSFKNASGIVEKRIIDPSLFSSGPVTDAAWRAACTNTSCGSASVSSFANTAGNVYYRSPSGSLLYDNNYVNTNCVLNIFSSLSGCSPSPAPSVASCGFHHHHHH

SEQ ID NO: 16 - DNA, 333 bp, Chryseobacterium defluvii
  CDS (1)..(333)
gctaccaatcaagatgtagttggaaaagaaaacaccagtaaccatgttgccgcaagggacttcggaaaaacggttcctgtgggaattaatgaagaaaacggaacgttgaaagtttctttcatccttagtgcccaattctacgaaattaagccaagcaaagaaaatgaagagtacatcagcctgatcaggcaggctatacagaatgagtctcctattcatgtttttatgaagcttaacagcaatgaaatcgtgaaggtggaaaaaggaactgaggaagatgttaaatactttaggtctatcctgaccaaggaagtaaaagaagaaaacaggaaa

SEQ ID NO: 17 - protein, 111 aa, Chryseobacterium defluvii
ATNQDVVGKENTSNHVAARDFGKTVPVGINEENGTLKVSFILSAQFYEIKPSKENEEYISLIRQAIQNESPIHVFMKLNSNEIVKVEKGTEEDVKYFRSILTKEVKEENRK

SEQ ID NO: 18 - DNA, 579 bp, Chryseobacterium defluvii
  CDS (1)..(579)
ttgacgagtgtacttcccaatgtaactactttaaacaatatgtttactcaaattaaaaaccagtcgtgcggaacttcaacagcttcttctccgtgtattacattcagatatgctgtagacggttgctacgcaagagctcacaaaatgagacaaatccttgtgaacaatggatatgattgtgaaaaacagtttatctatggaaatctaaaagcctctaccggttcttgctgtgtatcatggaattatcacgtagccattttggtgagctataaaaatgcttccggagttactgaaaaaagaattattgatccgtccctgtttcctaacgggcctgttactgaaactacctggagaaatgcgtgtgtaaatacctcttgcggaactgcatcctcttcttcttatgccaatacagcaggaaatatttattacagaagctcaaccggatcttatttgtatgataacagttacatcaataccaattgtgtactgacaacgttctcatcactttccggctgttctccgacaccggctccaagcgtatcacactgcggaggaatctctcatcatcaccatcaccac

SEQ ID NO: 19 - protein, 193 aa, Chryseobacterium defluvii
LTSVLPNVTTLNNMFTQIKNQSCGTSTASSPCITFRYAVDGCYARAHKMRQILVNNGYDCEKQFIYGNLKASTGSCCVSWNYHVAILVSYKNASGVTEKRIIDPSLFPNGPVTETTWRNACVNTSCGTASSSSYANTAGNIYYRSSTGSYLYDNSYINTNCVLTTFSSLSGCSPTPAPSVSHCGGISHHHHHH

SEQ ID NO: 20 - protein, 304 aa, Chryseobacterium defluvii
ATNQDVVGKENTSNHVAARDFGKTVPVGINEENGTLKVSFILSAQFYEIKPSKENEEYISLIRQAIQNESPIHVFMKLNSNEIVKVEKGTEEDVKYFRSILTKEVKEENRKLTSVLPNVTTLNNMFTQIKNQSCGTSTASSPCITFRYAVDGCYARAHKMRQILVNNGYDCEKQFIYGNLKASTGSCCVSWNYHVAILVSYKNASGVTEKRIIDPSLFPNGPVTETTWRNACVNTSCGTASSSSYANTAGNIYYRSSTGSYLYDNSYINTNCVLTTFSSLSGCSPTPAPSVSHCGGISHHHHHH

SEQ ID NO: 21 - protein, 8 aa, Artificial
  Amino acid sequence motif
DGCYARAH

SEQ ID NO: 22 - protein, 7 aa, Artificial
  Amino acid sequence motif
  MISC_FEATURE (7)..(7): Xaa is Arg or Lys or Gln
CYARAHX

SEQ ID NO: 23 - protein, 7 aa, Artificial
  Amino acid sequence motif
  MISC_FEATURE (4)..(4): Xaa is Leu or Val or Ile
HVAXLVS

SEQ ID NO: 24 - protein, 5 aa, Artificial
  Amino acid sequence motif
  MISC_FEATURE (1)..(1): Xaa is Ile or Met
  MISC_FEATURE (2)..(2): Xaa is Leu or Ile or Val
  MISC_FEATURE (3)..(3): Xaa is Ser or Thr
XXXAQ

SEQ ID NO: 25 - protein, 9 aa, Artificial
  Amino acid sequence motif
  MISC_FEATURE (1)..(1): Xaa is Lys or Arg
  MISC_FEATURE (2)..(2): Xaa is Val or Ile or Leu
  MISC_FEATURE (3)..(3): Xaa is Ser or Ala or Asn
  MISC_FEATURE (4)..(4): Xaa is any amino acid residue
  MISC_FEATURE (5)..(5): Xaa is Ile or Met
  MISC_FEATURE (6)..(6): Xaa is Leu or Ile or Val
  MISC_FEATURE (7)..(7): Xaa is Ser or Thr
XXXXXXXAQ